European Patent Application EP 4 166 144 A1, published April 19, 2023. Title: 双链siRNA类似物的缀合物. Applicant: 正大天晴药业集团股份有限公司 南京明德新药研发有限公司. The sequence listing filed with the application follows.

SEQUENCE LISTING (48 sequences)

SEQ ID NO: 1 - RNA, 19 nt, Artificial Sequence
  正义链
gugugcacuucgcuucaca

SEQ ID NO: 2 - RNA, 19 nt, Artificial Sequence
  反义链
ugugaagcgaagugcacac

SEQ ID NO: 3 - RNA, 18 nt, Artificial Sequence
  正义链
  modified_base (1)..(2): 核苷酸之间通过结构单元r以磷酸酯基连接
ggugcacuucgcuucaca

SEQ ID NO: 4 - RNA, 20 nt, Artificial Sequence
  反义链
  modified_base (5)..(6): 核苷酸之间通过结构单元r以磷酸酯基连接
ugugagcgaagugcacacuu

SEQ ID NO: 5 - RNA, 18 nt, Artificial Sequence
  正义链
  modified_base (2)..(3): 核苷酸之间通过结构单元r以磷酸酯基连接
guugcacuucgcuucaca

SEQ ID NO: 6 - RNA, 20 nt, Artificial Sequence
  反义链
  modified_base (1)..(2): 核苷酸之间通过结构单元r以磷酸酯基连接
uugaagcgaagugcacacuu

SEQ ID NO: 7 - RNA, 20 nt, Artificial Sequence
  反义链
  modified_base (2)..(3): 核苷酸之间通过结构单元r以磷酸酯基连接
uggaagcgaagugcacacuu

SEQ ID NO: 8 - RNA, 20 nt, Artificial Sequence
  反义链
  modified_base (3)..(4): 核苷酸之间通过结构单元r以磷酸酯基连接
uguaagcgaagugcacacuu

SEQ ID NO: 9 - RNA, 20 nt, Artificial Sequence
  反义链
  modified_base (4)..(5): 核苷酸之间通过结构单元r以磷酸酯基连接
ugugagcgaagugcacacuu

SEQ ID NO: 10 - RNA, 20 nt, Artificial Sequence
  反义链
  modified_base (6)..(7): 核苷酸之间通过结构单元r以磷酸酯基连接
ugugaacgaagugcacacuu

SEQ ID NO: 11 - RNA, 20 nt, Artificial Sequence
  反义链
  modified_base (7)..(8): 核苷酸之间通过结构单元r以磷酸酯基连接
ugugaaggaagugcacacuu

SEQ ID NO: 12 - RNA, 18 nt, Artificial Sequence
  正义链
  modified_base (6)..(7): 核苷酸之间通过结构单元r以磷酸酯基连接
gugugccuucgcuucaca

SEQ ID NO: 13 - RNA, 18 nt, Artificial Sequence
  正义链
  modified_base (16)..(17): 核苷酸之间通过结构单元r以磷酸酯基连接
gugugcacuucgcuucca

SEQ ID NO: 14 - RNA, 18 nt, Artificial Sequence
  正义链
  modified_base (17)..(17): 通过结构单元r以磷酸酯基连接
gugugcacuucgcuucac

SEQ ID NO: 15 - RNA, 18 nt, Artificial Sequence
  正义链
  modified_base (1)..(2): 硫代磷酸酯基连接
  modified_base (1)..(4): 甲氧基修饰
  modified_base (2)..(3): 硫代磷酸酯基连接
  modified_base (5)..(5): 氟代修饰
  modified_base (6)..(6): 甲氧基修饰
  modified_base (7)..(9): 氟代修饰
  modified_base (10)..(18): 甲氧基修饰
  modified_base (15)..(16): 核苷酸之间通过结构单元r以磷酸酯基连接
gugugcacuucgcuuaca

SEQ ID NO: 16 - RNA, 18 nt, Artificial Sequence
  正义链
  modified_base (1)..(2): 核苷酸之间通过结构单元r以硫代磷酸酯基连接
  modified_base (1)..(3): 甲氧基修饰
  modified_base (4)..(4): 氟代修饰
  modified_base (5)..(5): 甲氧基修饰
  modified_base (6)..(8): 氟代修饰
  modified_base (9)..(18): 甲氧基修饰
ggugcacuucgcuucaca

SEQ ID NO: 17 - RNA, 20 nt, Artificial Sequence
  反义链
  modified_base (1)..(2): 硫代磷酸酯基连接
  modified_base (1)..(1): 甲氧基修饰
  modified_base (2)..(3): 硫代磷酸酯基连接
  modified_base (2)..(2): 氟代修饰
  modified_base (3)..(6): 甲氧基修饰
  modified_base (5)..(6): 核苷酸之间通过结构单元r以磷酸酯基连接
  modified_base (7)..(8): 氟代修饰
  modified_base (9)..(12): 甲氧基修饰
  modified_base (13)..(13): 氟代修饰
  modified_base (14)..(14): 甲氧基修饰
  modified_base (15)..(15): 氟代修饰
  modified_base (16)..(20): 甲氧基修饰
  modified_base (18)..(19): 硫代磷酸酯基连接
  modified_base (19)..(20): 硫代磷酸酯基连接
ugugagcgaagugcacacuu

SEQ ID NO: 18 - RNA, 18 nt, Artificial Sequence
  正义链
  modified_base (1)..(2): 硫代磷酸酯基连接
  modified_base (2)..(3): 第2位核苷酸通过硫代磷酸酯基连接结构单元r，r与第3位核苷酸通过磷酸酯 基连接
  modified_base (4)..(4): 氟代修饰
  modified_base (5)..(5): 甲氧基修饰
  modified_base (6)..(8): 氟代修饰
  modified_base (9)..(18): 甲氧基修饰
guugcacuucgcuucaca

SEQ ID NO: 19 - RNA, 20 nt, Artificial Sequence
  反义链
  modified_base (1)..(2): 核苷酸之间通过结构单元r以硫代磷酸酯基连接
  modified_base (1)..(4): 甲氧基修饰
  modified_base (5)..(5): 氟代修饰
  modified_base (6)..(6): 甲氧基修饰
  modified_base (7)..(8): 氟代修饰
  modified_base (9)..(12): 甲氧基修饰
  modified_base (13)..(13): 氟代修饰
  modified_base (14)..(14): 甲氧基修饰
  modified_base (15)..(15): 氟代修饰
  modified_base (16)..(20): 甲氧基修饰
  modified_base (18)..(19): 通过硫代磷酸酯基连接
  modified_base (19)..(20): 通过硫代磷酸酯基连接
uugaagcgaagugcacacuu

SEQ ID NO: 20 - RNA, 20 nt, Artificial Sequence
  反义链
  modified_base (1)..(2): 硫代磷酸酯基连接
  modified_base (1)..(1): 甲氧基修饰
  modified_base (2)..(3): 第2位核苷酸通过硫代磷酸酯基连接结构单元r，r与第3位核苷酸通过磷酸酯 基连接
  modified_base (2)..(2): 氟代修饰
  modified_base (3)..(4): 甲氧基修饰
  modified_base (5)..(5): 氟代修饰
  modified_base (6)..(6): 甲氧基修饰
  modified_base (7)..(8): 氟代修饰
  modified_base (9)..(12): 甲氧基修饰
  modified_base (13)..(13): 氟代修饰
  modified_base (14)..(14): 甲氧基修饰
  modified_base (15)..(15): 氟代修饰
  modified_base (16)..(20): 甲氧基修饰
  modified_base (18)..(19): 硫代磷酸酯基连接
  modified_base (19)..(20): 硫代磷酸酯基连接
uggaagcgaagugcacacuu

SEQ ID NO: 21 - RNA, 20 nt, Artificial Sequence
  反义链
  modified_base (1)..(2): 硫代磷酸酯基连接
  modified_base (1)..(1): 甲氧基修饰
  modified_base (2)..(3): 硫代磷酸酯基连接
  modified_base (2)..(2): 氟代修饰
  modified_base (3)..(4): 核苷酸之间通过结构单元r以磷酸酯基连接
  modified_base (3)..(4): 甲氧基修饰
  modified_base (5)..(5): 氟代修饰
  modified_base (6)..(6): 甲氧基修饰
  modified_base (7)..(8): 氟代修饰
  modified_base (9)..(12): 甲氧基修饰
  modified_base (13)..(13): 氟代修饰
  modified_base (14)..(14): 甲氧基修饰
  modified_base (15)..(15): 氟代修饰
  modified_base (16)..(20): 甲氧基修饰
  modified_base (18)..(19): 硫代磷酸酯基连接
  modified_base (19)..(20): 硫代磷酸酯基连接
uguaagcgaagugcacacuu

SEQ ID NO: 22 - RNA, 20 nt, Artificial Sequence
  反义链
  modified_base (1)..(2): 硫代磷酸酯基连接
  modified_base (1)..(1): 甲氧基修饰
  modified_base (2)..(3): 硫代磷酸酯基连接
  modified_base (2)..(2): 氟代修饰
  modified_base (3)..(4): 甲氧基修饰
  modified_base (4)..(5): 核苷酸之间通过结构单元r以磷酸酯基连接
  modified_base (5)..(5): 氟代修饰
  modified_base (6)..(6): 甲氧基修饰
  modified_base (7)..(8): 氟代修饰
  modified_base (9)..(12): 甲氧基修饰
  modified_base (13)..(13): 氟代修饰
  modified_base (14)..(14): 甲氧基修饰
  modified_base (15)..(15): 氟代修饰
  modified_base (16)..(20): 甲氧基修饰
  modified_base (18)..(19): 硫代磷酸酯基连接
  modified_base (19)..(20): 硫代磷酸酯基连接
ugugagcgaagugcacacuu

SEQ ID NO: 23 - RNA, 20 nt, Artificial Sequence
  反义链
  modified_base (1)..(2): 硫代磷酸酯基连接
  modified_base (1)..(1): 甲氧基修饰
  modified_base (2)..(3): 硫代磷酸酯基连接
  modified_base (2)..(2): 氟代修饰
  modified_base (3)..(5): 甲氧基修饰
  modified_base (6)..(7): 核苷酸之间通过磷酸酯基连接结构单元r
  modified_base (6)..(8): 氟代修饰
  modified_base (9)..(12): 甲氧基修饰
  modified_base (13)..(13): 氟代修饰
  modified_base (14)..(14): 甲氧基修饰
  modified_base (15)..(15): 氟代修饰
  modified_base (16)..(20): 甲氧基修饰
  modified_base (18)..(19): 硫代磷酸酯基连接
  modified_base (19)..(20): 硫代磷酸酯基连接
ugugaacgaagugcacacuu

SEQ ID NO: 24 - RNA, 20 nt, Artificial Sequence
  反义链
  modified_base (1)..(2): 硫代磷酸酯基连接
  modified_base (1)..(1): 甲氧基修饰
  modified_base (2)..(3): 硫代磷酸酯基连接
  modified_base (2)..(2): 氟代修饰
  modified_base (3)..(5): 甲氧基修饰
  modified_base (6)..(6): 氟代修饰
  modified_base (7)..(8): 核苷酸之间通过结构单元r以磷酸酯基连接
  modified_base (7)..(7): 甲氧基修饰
  modified_base (8)..(8): 氟代修饰
  modified_base (9)..(12): 甲氧基修饰
  modified_base (13)..(13): 氟代修饰
  modified_base (14)..(14): 甲氧基修饰
  modified_base (15)..(15): 氟代修饰
  modified_base (16)..(20): 甲氧基修饰
  modified_base (18)..(19): 硫代磷酸酯基连接
  modified_base (19)..(20): 硫代磷酸酯基连接
ugugaaggaagugcacacuu

SEQ ID NO: 25 - RNA, 18 nt, Artificial Sequence
  正义链
  modified_base (1)..(2): 硫代磷酸酯基连接
  modified_base (1)..(4): 甲氧基修饰
  modified_base (2)..(3): 硫代磷酸酯基连接
  modified_base (5)..(5): 甲氧基修饰
  modified_base (6)..(7): 核苷酸之间通过结构单元r以磷酸酯基连接
  modified_base (6)..(6): 甲氧基修饰
  modified_base (7)..(8): 氟代修饰
  modified_base (9)..(18): 甲氧基修饰
gugugccuucgcuucaca

SEQ ID NO: 26 - RNA, 18 nt, Artificial Sequence
  正义链
  modified_base (1)..(2): 硫代磷酸酯基连接
  modified_base (1)..(4): 甲氧基修饰
  modified_base (2)..(3): 硫代磷酸酯基连接
  modified_base (5)..(5): 氟代修饰
  modified_base (6)..(6): 甲氧基修饰
  modified_base (7)..(9): 氟代修饰
  modified_base (10)..(18): 甲氧基修饰
  modified_base (16)..(17): 核苷酸之间通过结构单元r以磷酸酯基连接
gugugcacuucgcuucca

SEQ ID NO: 27 - RNA, 18 nt, Artificial Sequence
  正义链
  modified_base (1)..(2): 硫代磷酸酯基连接
  modified_base (1)..(4): 甲氧基修饰
  modified_base (2)..(3): 硫代磷酸酯基连接
  modified_base (5)..(5): 氟代修饰
  modified_base (6)..(6): 甲氧基修饰
  modified_base (7)..(9): 氟代修饰
  modified_base (10)..(18): 甲氧基修饰
  modified_base (18)..(18): 通过磷酸酯基连接结构单元r
gugugcacuucgcuucac

SEQ ID NO: 28 - RNA, 19 nt, Artificial Sequence
  正义链
  modified_base (1)..(2): 硫代磷酸酯基连接
  modified_base (1)..(4): 甲氧基修饰
  modified_base (2)..(3): 硫代磷酸酯基连接
  modified_base (5)..(5): 氟代修饰
  modified_base (6)..(6): 甲氧基修饰
  modified_base (7)..(9): 氟代修饰
  modified_base (10)..(19): 甲氧基修饰
gugugcacuucgcuucaca

SEQ ID NO: 29 - RNA, 20 nt, Artificial Sequence
  反义链
  modified_base (9)..(10): 核苷酸之间通过结构单元r以磷酸酯基连接
ugugaagcgagugcacacuu

SEQ ID NO: 30 - RNA, 20 nt, Artificial Sequence
  反义链
  modified_base (10)..(11): 核苷酸之间通过结构单元r以磷酸酯基连接
ugugaagcgagugcacacuu

SEQ ID NO: 31 - RNA, 20 nt, Artificial Sequence
  反义链
  modified_base (15)..(16): 核苷酸之间通过结构单元r以磷酸酯基连接
ugugaagcgaagugccacuu

SEQ ID NO: 32 - RNA, 20 nt, Artificial Sequence
  反义链
  modified_base (17)..(18): 核苷酸之间通过结构单元r以磷酸酯基连接
ugugaagcgaagugcaccuu

SEQ ID NO: 33 - RNA, 19 nt, Artificial Sequence
  反义链
  modified_base (1)..(2): 硫代磷酸酯基连接
  modified_base (1)..(1): 甲氧基修饰
  modified_base (2)..(3): 硫代磷酸酯基连接
  modified_base (2)..(2): 氟代修饰
  modified_base (3)..(6): 甲氧基修饰
  modified_base (5)..(5): 通过磷酸酯基连接(Agn)残基
  modified_base (7)..(8): 氟代修饰
  modified_base (8)..(9): 核苷酸之间通过结构单元r以磷酸酯基连接
  modified_base (9)..(11): 甲氧基修饰
  modified_base (12)..(12): 氟代修饰
  modified_base (13)..(13): 甲氧基修饰
  modified_base (14)..(14): 氟代修饰
  modified_base (15)..(19): 甲氧基修饰
  modified_base (17)..(18): 硫代磷酸酯基连接
  modified_base (18)..(19): 硫代磷酸酯基连接
ugugagcgagugcacacuu

SEQ ID NO: 34 - RNA, 19 nt, Artificial Sequence
  反义链
  modified_base (1)..(2): 通过硫代磷酸酯基连接
  modified_base (1)..(1): 甲氧基修饰
  modified_base (2)..(3): 通过硫代磷酸酯基连接
  modified_base (2)..(2): 氟代修饰
  modified_base (3)..(6): 甲氧基修饰
  modified_base (5)..(5): 通过磷酸酯基连接(Agn)残基
  modified_base (7)..(8): 氟代修饰
  modified_base (9)..(10): 核苷酸之间通过结构单元r以磷酸酯基连接
  modified_base (9)..(11): 甲氧基修饰
  modified_base (12)..(12): 氟代修饰
  modified_base (13)..(13): 甲氧基修饰
  modified_base (14)..(14): 氟代修饰
  modified_base (15)..(19): 甲氧基修饰
  modified_base (17)..(18): 通过硫代磷酸酯基连接
  modified_base (18)..(19): 通过硫代磷酸酯基连接
ugugagcgagugcacacuu

SEQ ID NO: 35 - RNA, 19 nt, Artificial Sequence
  反义链
  modified_base (1)..(2): 硫代磷酸酯基连接
  modified_base (1)..(1): 甲氧基修饰
  modified_base (2)..(3): 硫代磷酸酯基连接
  modified_base (2)..(2): 氟代修饰
  modified_base (3)..(6): 甲氧基修饰
  modified_base (5)..(5): 通过磷酸酯基连接(Agn)残基
  modified_base (7)..(8): 氟代修饰
  modified_base (9)..(12): 甲氧基修饰
  modified_base (13)..(13): 氟代修饰
  modified_base (14)..(15): 核苷酸之间通过结构单元r以磷酸酯基连接
  modified_base (14)..(19): 甲氧基修饰
  modified_base (17)..(18): 硫代磷酸酯基连接
  modified_base (18)..(19): 硫代磷酸酯基连接
ugugagcgaagugccacuu

SEQ ID NO: 36 - RNA, 19 nt, Artificial Sequence
  反义链
  modified_base (1)..(2): 硫代磷酸酯基连接
  modified_base (1)..(1): 甲氧基修饰
  modified_base (2)..(3): 硫代磷酸酯基连接
  modified_base (2)..(2): 氟代修饰
  modified_base (3)..(6): 甲氧基修饰
  modified_base (5)..(5): 通过磷酸酯基连接(Agn)残基
  modified_base (7)..(8): 氟代修饰
  modified_base (9)..(12): 甲氧基修饰
  modified_base (13)..(13): 氟代修饰
  modified_base (14)..(14): 甲氧基修饰
  modified_base (15)..(15): 氟代修饰
  modified_base (16)..(17): 核苷酸之间通过结构单元r以磷酸酯基连接
  modified_base (16)..(19): 甲氧基修饰
  modified_base (17)..(18): 硫代磷酸酯基连接
  modified_base (18)..(19): 硫代磷酸酯基连接
ugugagcgaagugcaccuu

SEQ ID NO: 37 - RNA, 17 nt, Artificial Sequence
  正义链
  modified_base (1)..(2): 核苷酸之间通过结构单元r以磷酸酯基连接
  modified_base (13)..(14): 核苷酸之间通过结构单元r以磷酸酯基连接
ggugcacuucgcucaca

SEQ ID NO: 38 - RNA, 17 nt, Artificial Sequence
  正义链
  modified_base (1)..(2): 核苷酸之间通过结构单元r以磷酸酯基连接
  modified_base (10)..(11): 核苷酸之间通过结构单元r以磷酸酯基连接
ggugcacuuccuucaca

SEQ ID NO: 39 - RNA, 19 nt, Artificial Sequence
  反义链
  modified_base (3)..(4): 核苷酸之间通过结构单元r以磷酸酯基连接
  modified_base (5)..(6): 核苷酸之间通过结构单元r以磷酸酯基连接
uguaacgaagugcacacuu

SEQ ID NO: 40 - RNA, 20 nt, Artificial Sequence
  反义链
  modified_base (11)..(12): 核苷酸之间通过结构单元r以磷酸酯基连接
ugugaagcgaaugcacacuu

SEQ ID NO: 41 - RNA, 19 nt, Artificial Sequence
  反义链
  modified_base (1)..(1): (E)-乙烯基磷酸酯修饰的核苷酸
  modified_base (1)..(2): 硫代磷酸酯基连接
  modified_base (1)..(1): 甲氧基修饰
  modified_base (2)..(3): 硫代磷酸酯基连接
  modified_base (2)..(2): 氟代修饰
  modified_base (3)..(6): 甲氧基修饰
  modified_base (5)..(5): 通过磷酸酯基连接(Agn)残基
  modified_base (7)..(8): 氟代修饰
  modified_base (9)..(10): 核苷酸之间通过结构单元r以磷酸酯基连接
  modified_base (9)..(11): 甲氧基修饰
  modified_base (12)..(12): 氟代修饰
  modified_base (13)..(13): 甲氧基修饰
  modified_base (14)..(14): 氟代修饰
  modified_base (15)..(19): 甲氧基修饰
  modified_base (17)..(18): 硫代磷酸酯基连接
  modified_base (18)..(19): 硫代磷酸酯基连接
ugugagcgagugcacacuu

SEQ ID NO: 42 - RNA, 17 nt, Artificial Sequence
  正义链
  modified_base (1)..(2): 核苷酸之间通过结构单元r以硫代磷酸酯基连接
  modified_base (1)..(3): 甲氧基修饰
  modified_base (4)..(4): 氟代修饰
  modified_base (5)..(5): 甲氧基修饰
  modified_base (6)..(8): 氟代修饰
  modified_base (9)..(17): 甲氧基修饰
  modified_base (13)..(14): 核苷酸之间通过结构单元r以磷酸酯基连接
ggugcacuucgcucaca

SEQ ID NO: 43 - RNA, 17 nt, Artificial Sequence
  正义链
  modified_base (1)..(2): 核苷酸之间通过结构单元r以磷酸酯基连接
  modified_base (1)..(3): 甲氧基修饰
  modified_base (4)..(4): 氟代修饰
  modified_base (5)..(5): 甲氧基修饰
  modified_base (6)..(8): 氟代修饰
  modified_base (9)..(17): 甲氧基修饰
  modified_base (10)..(11): 核苷酸之间通过结构单元r以磷酸酯基连接
ggugcacuuccuucaca

SEQ ID NO: 44 - RNA, 19 nt, Artificial Sequence
  反义链
  modified_base (1)..(2): 硫代磷酸酯基连接
  modified_base (1)..(1): 甲氧基修饰
  modified_base (2)..(3): 硫代磷酸酯基连接
  modified_base (2)..(2): 氟代修饰
  modified_base (3)..(4): 核苷酸之间通过结构单元r以磷酸酯基连接
  modified_base (3)..(4): 甲氧基修饰
  modified_base (5)..(6): 核苷酸之间通过结构单元r以磷酸酯基连接
  modified_base (5)..(7): 氟代修饰
  modified_base (8)..(11): 甲氧基修饰
  modified_base (12)..(12): 氟代修饰
  modified_base (13)..(13): 甲氧基修饰
  modified_base (14)..(14): 氟代修饰
  modified_base (15)..(19): 甲氧基修饰
  modified_base (17)..(18): 硫代磷酸酯基连接
  modified_base (18)..(19): 硫代磷酸酯基连接
uguaacgaagugcacacuu

SEQ ID NO: 45 - RNA, 19 nt, Artificial Sequence
  反义链
  modified_base (1)..(2): 硫代磷酸酯基连接
  modified_base (1)..(1): 甲氧基修饰
  modified_base (2)..(3): 硫代磷酸酯基连接
  modified_base (2)..(2): 氟代修饰
  modified_base (3)..(5): 甲氧基修饰
  modified_base (5)..(5): 通过磷酸酯基连接(Agn)残基
  modified_base (5)..(6): 核苷酸之间通过结构单元r以磷酸酯基连接
  modified_base (6)..(7): 氟代修饰
  modified_base (8)..(11): 甲氧基修饰
  modified_base (12)..(12): 氟代修饰
  modified_base (13)..(13): 甲氧基修饰
  modified_base (14)..(14): 氟代修饰
  modified_base (15)..(19): 甲氧基修饰
  modified_base (17)..(18): 硫代磷酸酯基连接
  modified_base (18)..(19): 硫代磷酸酯基连接
ugugacgaagugcacacuu

SEQ ID NO: 46 - RNA, 19 nt, Artificial Sequence
  反义链
  modified_base (1)..(2): 硫代磷酸酯基连接
  modified_base (1)..(1): 甲氧基修饰
  modified_base (2)..(3): 硫代磷酸酯基连接
  modified_base (2)..(2): 氟代修饰
  modified_base (3)..(6): 甲氧基修饰
  modified_base (5)..(5): 通过磷酸酯基连接(Agn)残基
  modified_base (7)..(8): 氟代修饰
  modified_base (9)..(11): 甲氧基修饰
  modified_base (10)..(11): 核苷酸之间通过结构单元r以磷酸酯基连接
  modified_base (12)..(12): 氟代修饰
  modified_base (13)..(13): 甲氧基修饰
  modified_base (14)..(14): 氟代修饰
  modified_base (15)..(19): 甲氧基修饰
  modified_base (17)..(18): 硫代磷酸酯基连接
  modified_base (18)..(19): 硫代磷酸酯基连接
ugugagcgaaugcacacuu

SEQ ID NO: 47 - RNA, 20 nt, Artificial Sequence
  反义链
  modified_base (1)..(1): (E)-乙烯基磷酸酯修饰
  modified_base (1)..(2): 硫代磷酸酯基连接
  modified_base (1)..(1): 甲氧基修饰
  modified_base (2)..(3): 硫代磷酸酯基连接
  modified_base (2)..(2): 氟代修饰
  modified_base (3)..(5): 甲氧基修饰
  modified_base (6)..(7): 核苷酸之间通过结构单元r以磷酸酯基连接
  modified_base (6)..(8): 氟代修饰
  modified_base (9)..(12): 甲氧基修饰
  modified_base (13)..(13): 氟代修饰
  modified_base (14)..(14): 甲氧基修饰
  modified_base (15)..(15): 氟代修饰
  modified_base (16)..(20): 甲氧基修饰
  modified_base (18)..(19): 硫代磷酸酯基连接
  modified_base (19)..(20): 硫代磷酸酯基连接
ugugaacgaagugcacacuu

SEQ ID NO: 48 - RNA, 19 nt, Artificial Sequence
  反义链
  modified_base (1)..(1): (E)-乙烯基磷酸酯修饰
  modified_base (1)..(2): 硫代磷酸酯基连接
  modified_base (1)..(1): 甲氧基修饰
  modified_base (2)..(3): 硫代磷酸酯基连接
  modified_base (2)..(2): 氟代修饰
  modified_base (3)..(5): 甲氧基修饰
  modified_base (5)..(5): 通过磷酸酯基连接(Agn)残基
  modified_base (5)..(6): 核苷酸之间通过结构单元r以磷酸酯基连接
  modified_base (6)..(7): 氟代修饰
  modified_base (8)..(11): 甲氧基修饰
  modified_base (12)..(12): 氟代修饰
  modified_base (13)..(13): 甲氧基修饰
  modified_base (14)..(14): 氟代修饰
  modified_base (15)..(19): 甲氧基修饰
  modified_base (17)..(18): 硫代磷酸酯基连接
  modified_base (18)..(19): 硫代磷酸酯基连接
ugugacgaagugcacacuu